European Patent Specification EP 3 392 276 B1, published April 19, 2023. Title: HETERODIMER MOLECULE BASED ON CH3 STRUCTURAL DOMAIN, AND PREPARATION METHOD THEREFOR AND USE THEREOF. Applicant: SUZHOU ALPHAMAB CO., LTD. The sequence listing filed with the application follows.

SEQUENCE LISTING (36 sequences)

SEQ ID NO: 1 - protein, 227 aa, Homo sapiens
DKTHTCPPCPAPELLGGPSVFLFPPKPKDTLMISRTPEVTCVVVDVSHEDPEVKFNWYVDGVEVHNAKTKPREEQYNSTYRVVSVLTVLHQDWLNGKEYKCKVSNKALPAPIEKTISKAKGQPREPQVYTLPPSRDELTKNQVSLTCLVKGFYPSDIAVEWESNGQPENNYKTTPPVLDSDGSFFLYSKLTVDKSRWQQGNVFSCSVMHEALHNHYTQKSLSLSPGK

SEQ ID NO: 2 - DNA, 681 bp, Homo sapiens
gacaagacccacacctgccccccctgccccgcccccgagctgctgggcggccccagcgtgttcctgttcccccccaagcccaaggacaccctgatgatcagccgcacccccgaggtgacctgcgtggtggtggacgtgagccacgagaaccccgaggtgaagttcaactggtacgtggacggcgtggaggtgcacaacgccaagaccaagccccgcgaggagcagtacaacagcacctaccgcgtggtgagcgtgctgaccgtgctgcaccaggactggctgaacggcaaggagtacaagtgcaaggtgagcaacaaggccctgcccgcccccatcgagaagaccatcagcaaggccaagggccagccccgcgagccccaggtgtacaccctgccccccagccgcgacgagctgaccaagaaccaggtgagcctgacctgcctggtgaagggcttctaccccagcgacatcgccgtggagtgggagagcaacggccagcccgagaacaactacaagaccaccccccccgtgctggacagcgacggcagcttcttcctgtacagcaagctgaccgtggacaagagccgctggcagcagggcaacgtgttcagctgcagcgtgatgcacgaggccctgcacaaccactacacccagaagagcctgagcctgagccccggcaag

SEQ ID NO: 3 - DNA, 741 bp, artificial sequence
  kappaIII signal peptide
atggagaccgacaccctgctgctgtgggtgctgctgctgtgggtgcccggcagcaccggcgacaagacccacacctgccccccctgccccgcccccgagctgctgggcggccccagcgtgttcctgttcccccccaagcccaaggacaccctgatgatcagccgcacccccgaggtgacctgcgtggtggtggacgtgagccacgagaaccccgaggtgaagttcaactggtacgtggacggcgtggaggtgcacaacgccaagaccaagccccgcgaggagcagtacaacagcacctaccgcgtggtgagcgtgctgaccgtgctgcaccaggactggctgaacggcaaggagtacaagtgcaaggtgagcaacaaggccctgcccgcccccatcgagaagaccatcagcaaggccaagggccagccccgcgagccccaggtgtacaccctgccccccagccgcgacgagctgaccaagaaccaggtgagcctgacctgcctggtgaagggcttctaccccagcgacatcgccgtggagtgggagagcaacggccagcccgagaacaactacaagaccaccccccccgtgctggacagcgacggcagcttcttcctgtacagcaagctgaccgtggacaagagccgctggcagcagggcaacgtgttcagctgcagcgtgatgcacgaggccctgcacaaccactacacccagaagagcctgagcctgagccccggcaag

SEQ ID NO: 4 - protein, 471 aa, artificial sequence
  a ScFv-Fc fusion protein
EVQLLESGGGVVQPGRSLRLSCIASGFTFSSYPMTWVRQAPGKGLEWVASISYDGSYKYKADSMKGRLTISRDNSKNTLYLEMNSLTAEDTAVYYCARTAFFNAYDFWGQGTLVTVSSASTKGPSVGGGGSGGGGSEIVMTQSPATLSVSPGERATLSCRASQSVRSNLAWYQQKPGQAPRLLIYAASTRATGIPARFSGSGSGTEFTLTISSLQSEDFAVYYCQQYNEWFRTSGQGTKVEIKRDKTHTCPPCPAPELLGGPSVFLFPPKPKDTLMISRTPEVTCVVVDVSHENPEVKFNWYVDGVEVHNAKTKPREEQYNSTYRVVSVLTVLHQDWLNGKEYKCKVSNKALPAPIEKTISKAKGQPREPQVYTLPPSRDELTKNQVSLTCLVKGFYPSDIAVEWESNGQPENNYKTTPPVLDSDGSFFLYSKLTVDKSRWQQGNVFSCSVMHEALHNHYTQKSLSLSPGK

SEQ ID NO: 5 - DNA, 1473 bp, artificial sequence
  ScFv-Fc fusion protein coding gene
atggagaccgacaccctgctgctgtgggtgctgctgctgtgggtgcccggcagcaccggcgaggtgcagctgctggagagcggcggcggcgtggtgcagcccggccgcagcctgcgcctgagctgcatcgccagcggcttcaccttcagcagctaccccatgacctgggtgcgccaggcccccggcaagggcctggagtgggtggccagcatcagctacgacggcagctacaagtacaaggccgacagcatgaagggccgcctgaccatcagccgcgacaacagcaagaacaccctgtacctggagatgaacagcctgaccgccgaggacaccgccgtgtactactgcgcccgcaccgccttcttcaacgcctacgacttctggggccagggcaccctggtgaccgtgagcagcgccagcaccaagggccccagcgtgggcggcggcggcagcggcggcggcggcagcgagatcgtgatgacccagagccccgccaccctgagcgtgagccccggcgagcgcgccaccctgagctgccgcgccagccagagcgtgcgcagcaacctggcctggtaccagcagaagcccggccaggccccccgcctgctgatctacgccgccagcacccgcgccaccggcatccccgcccgcttcagcggcagcggcagcggcaccgagttcaccctgaccatcagcagcctgcagagcgaggacttcgccgtgtactactgccagcagtacaacgagtggttccgcaccagcggccagggcaccaaggtggagatcaagcgcgacaagacccacacctgccccccctgccccgcccccgagctgctgggcggccccagcgtgttcctgttcccccccaagcccaaggacaccctgatgatcagccgcacccccgaggtgacctgcgtggtggtggacgtgagccacgagaaccccgaggtgaagttcaactggtacgtggacggcgtggaggtgcacaacgccaagaccaagccccgcgaggagcagtacaacagcacctaccgcgtggtgagcgtgctgaccgtgctgcaccaggactggctgaacggcaaggagtacaagtgcaaggtgagcaacaaggccctgcccgcccccatcgagaagaccatcagcaaggccaagggccagccccgcgagccccaggtgtacaccctgccccccagccgcgacgagctgaccaagaaccaggtgagcctgacctgcctggtgaagggcttctaccccagcgacatcgccgtggagtgggagagcaacggccagcccgagaacaactacaagaccaccccccccgtgctggacagcgacggcagcttcttcctgtacagcaagctgaccgtggacaagagccgctggcagcagggcaacgtgttcagctgcagcgtgatgcacgaggccctgcacaaccactacacccagaagagcctgagcctgagccccggcaag

SEQ ID NO: 6 - protein, 471 aa, artificial sequence
  Y349C+T366W
EVQLLESGGGVVQPGRSLRLSCIASGFTFSSYPMTWVRQAPGKGLEWVASISYDGSYKYKADSMKGRLTISRDNSKNTLYLEMNSLTAEDTAVYYCARTAFFNAYDFWGQGTLVTVSSASTKGPSVGGGGSGGGGSEIVMTQSPATLSVSPGERATLSCRASQSVRSNLAWYQQKPGQAPRLLIYAASTRATGIPARFSGSGSGTEFTLTISSLQSEDFAVYYCQQYNEWFRTSGQGTKVEIKRDKTHTCPPCPAPELLGGPSVFLFPPKPKDTLMISRTPEVTCVVVDVSHENPEVKFNWYVDGVEVHNAKTKPREEQYNSTYRVVSVLTVLHQDWLNGKEYKCKVSNKALPAPIEKTISKAKGQPREPQVCTLPPSRDELTKNQVSLWCLVKGFYPSDIAVEWESNGQPENNYKTTPPVLDSDGSFFLYSKLTVDKSRWQQGNVFSCSVMHEALHNHYTQKSLSLSPGK

SEQ ID NO: 7 - protein, 227 aa, artificial sequence
  D356C+T366S+L368A+Y407V
DKTHTCPPCPAPELLGGPSVFLFPPKPKDTLMISRTPEVTCVVVDVSHEDPEVKFNWYVDGVEVHNAKTKPREEQYNSTYRVVSVLTVLHQDWLNGKEYKCKVSNKALPAPIEKTISKAKGQPREPQVYTLPPSRCELTKNQVSLSCAVKGFYPSDIAVEWESNGQPENNYKTTPPVLDSDGSFFLVSKLTVDKSRWQQGNVFSCSVMHEALHNHYTQKSLSLSPGK

SEQ ID NO: 8 - protein, 227 aa, artificial sequence
  D356C+T366S+L368A+Y407V+F405K
DKTHTCPPCPAPELLGGPSVFLFPPKPKDTLMISRTPEVTCVVVDVSHEDPEVKFNWYVDGVEVHNAKTKPREEQYNSTYRVVSVLTVLHQDWLNGKEYKCKVSNKALPAPIEKTISKAKGQPREPQVYTLPPSRCELTKNQVSLSCAVKGFYPSDIAVEWESNGQPENNYKTTPPVLDSDGSFKLVSKLTVDKSRWQQGNVFSCSVMHEALHNHYTQKSLSLSPGK

SEQ ID NO: 9 - protein, 471 aa, artificial sequence
  Y349C+T366W+F405K
EVQLLESGGGVVQPGRSLRLSCIASGFTFSSYPMTWVRQAPGKGLEWVASISYDGSYKYKADSMKGRLTISRDNSKNTLYLEMNSLTAEDTAVYYCARTAFFNAYDFWGQGTLVTVSSASTKGPSVGGGGSGGGGSEIVMTQSPATLSVSPGERATLSCRASQSVRSNLAWYQQKPGQAPRLLIYAASTRATGIPARFSGSGSGTEFTLTISSLQSEDFAVYYCQQYNEWFRTSGQGTKVEIKRDKTHTCPPCPAPELLGGPSVFLFPPKPKDTLMISRTPEVTCVVVDVSHENPEVKFNWYVDGVEVHNAKTKPREEQYNSTYRVVSVLTVLHQDWLNGKEYKCKVSNKALPAPIEKTISKAKGQPREPQVCTLPPSRDELTKNQVSLWCLVKGFYPSDIAVEWESNGQPENNYKTTPPVLDSDGSFKLYSKLTVDKSRWQQGNVFSCSVMHEALHNHYTQKSLSLSPGK

SEQ ID NO: 10 - protein, 471 aa, artificial sequence
  Y349C+T366W+K409E
EVQLLESGGGVVQPGRSLRLSCIASGFTFSSYPMTWVRQAPGKGLEWVASISYDGSYKYKADSMKGRLTISRDNSKNTLYLEMNSLTAEDTAVYYCARTAFFNAYDFWGQGTLVTVSSASTKGPSVGGGGSGGGGSEIVMTQSPATLSVSPGERATLSCRASQSVRSNLAWYQQKPGQAPRLLIYAASTRATGIPARFSGSGSGTEFTLTISSLQSEDFAVYYCQQYNEWFRTSGQGTKVEIKRDKTHTCPPCPAPELLGGPSVFLFPPKPKDTLMISRTPEVTCVVVDVSHENPEVKFNWYVDGVEVHNAKTKPREEQYNSTYRVVSVLTVLHQDWLNGKEYKCKVSNKALPAPIEKTISKAKGQPREPQVCTLPPSRDELTKNQVSLWCLVKGFYPSDIAVEWESNGQPENNYKTTPPVLDSDGSFFLYSELTVDKSRWQQGNVFSCSVMHEALHNHYTQKSLSLSPGK

SEQ ID NO: 11 - protein, 471 aa, artificial sequence
  Y349C+T366W+K409A
EVQLLESGGGVVQPGRSLRLSCIASGFTFSSYPMTWVRQAPGKGLEWVASISYDGSYKYKADSMKGRLTISRDNSKNTLYLEMNSLTAEDTAVYYCARTAFFNAYDFWGQGTLVTVSSASTKGPSVGGGGSGGGGSEIVMTQSPATLSVSPGERATLSCRASQSVRSNLAWYQQKPGQAPRLLIYAASTRATGIPARFSGSGSGTEFTLTISSLQSEDFAVYYCQQYNEWFRTSGQGTKVEIKRDKTHTCPPCPAPELLGGPSVFLFPPKPKDTLMISRTPEVTCVVVDVSHENPEVKFNWYVDGVEVHNAKTKPREEQYNSTYRVVSVLTVLHQDWLNGKEYKCKVSNKALPAPIEKTISKAKGQPREPQVCTLPPSRDELTKNQVSLWCLVKGFYPSDIAVEWESNGQPENNYKTTPPVLDSDGSFFLYSALTVDKSRWQQGNVFSCSVMHEALHNHYTQKSLSLSPGK

SEQ ID NO: 12 - protein, 471 aa, artificial sequence
  Y349C+T366W+F405K+K360E+Q347E
EVQLLESGGGVVQPGRSLRLSCIASGFTFSSYPMTWVRQAPGKGLEWVASISYDGSYKYKADSMKGRLTISRDNSKNTLYLEMNSLTAEDTAVYYCARTAFFNAYDFWGQGTLVTVSSASTKGPSVGGGGSGGGGSEIVMTQSPATLSVSPGERATLSCRASQSVRSNLAWYQQKPGQAPRLLIYAASTRATGIPARFSGSGSGTEFTLTISSLQSEDFAVYYCQQYNEWFRTSGQGTKVEIKRDKTHTCPPCPAPELLGGPSVFLFPPKPKDTLMISRTPEVTCVVVDVSHENPEVKFNWYVDGVEVHNAKTKPREEQYNSTYRVVSVLTVLHQDWLNGKEYKCKVSNKALPAPIEKTISKAKGQPREPEVCTLPPSRDELTENQVSLWCLVKGFYPSDIAVEWESNGQPENNYKTTPPVLDSDGSFKLYSKLTVDKSRWQQGNVFSCSVMHEALHNHYTQKSLSLSPGK

SEQ ID NO: 13 - protein, 227 aa, artificial sequence
  D356C+T366S+L368A+Y407V+Q347R
DKTHTCPPCPAPELLGGPSVFLFPPKPKDTLMISRTPEVTCVVVDVSHEDPEVKFNWYVDGVEVHNAKTKPREEQYNSTYRVVSVLTVLHQDWLNGKEYKCKVSNKALPAPIEKTISKAKGQPREPRVYTLPPSRCELTKNQVSLSCAVKGFYPSDIAVEWESNGQPENNYKTTPPVLDSDGSFFLVSKLTVDKSRWQQGNVFSCSVMHEALHNHYTQKSLSLSPGK

SEQ ID NO: 14 - protein, 471 aa, artificial sequence
  Y349C+T366W+F405K+Q347R
EVQLLESGGGVVQPGRSLRLSCIASGFTFSSYPMTWVRQAPGKGLEWVASISYDGSYKYKADSMKGRLTISRDNSKNTLYLEMNSLTAEDTAVYYCARTAFFNAYDFWGQGTLVTVSSASTKGPSVGGGGSGGGGSEIVMTQSPATLSVSPGERATLSCRASQSVRSNLAWYQQKPGQAPRLLIYAASTRATGIPARFSGSGSGTEFTLTISSLQSEDFAVYYCQQYNEWFRTSGQGTKVEIKRDKTHTCPPCPAPELLGGPSVFLFPPKPKDTLMISRTPEVTCVVVDVSHENPEVKFNWYVDGVEVHNAKTKPREEQYNSTYRVVSVLTVLHQDWLNGKEYKCKVSNKALPAPIEKTISKAKGQPREPRVCTLPPSRDELTKNQVSLWCLVKGFYPSDIAVEWESNGQPENNYKTTPPVLDSDGSFKLYSKLTVDKSRWQQGNVFSCSVMHEALHNHYTQKSLSLSPGK

SEQ ID NO: 15 - protein, 227 aa, artificial sequence
  D356C+T366S+L368A+Y407V+K360E+Q347E
DKTHTCPPCPAPELLGGPSVFLFPPKPKDTLMISRTPEVTCVVVDVSHEDPEVKFNWYVDGVEVHNAKTKPREEQYNSTYRVVSVLTVLHQDWLNGKEYKCKVSNKALPAPIEKTISKAKGQPREPEVYTLPPSRCELTENQVSLSCAVKGFYPSDIAVEWESNGQPENNYKTTPPVLDSDGSFFLVSKLTVDKSRWQQGNVFSCSVMHEALHNHYTQKSLSLSPGK

SEQ ID NO: 16 - protein, 471 aa, artificial sequence
  Y349C+T366W+K409A+K360E+Q347E
EVQLLESGGGVVQPGRSLRLSCIASGFTFSSYPMTWVRQAPGKGLEWVASISYDGSYKYKADSMKGRLTISRDNSKNTLYLEMNSLTAEDTAVYYCARTAFFNAYDFWGQGTLVTVSSASTKGPSVGGGGSGGGGSEIVMTQSPATLSVSPGERATLSCRASQSVRSNLAWYQQKPGQAPRLLIYAASTRATGIPARFSGSGSGTEFTLTISSLQSEDFAVYYCQQYNEWFRTSGQGTKVEIKRDKTHTCPPCPAPELLGGPSVFLFPPKPKDTLMISRTPEVTCVVVDVSHENPEVKFNWYVDGVEVHNAKTKPREEQYNSTYRVVSVLTVLHQDWLNGKEYKCKVSNKALPAPIEKTISKAKGQPREPEVCTLPPSRDELTENQVSLWCLVKGFYPSDIAVEWESNGQPENNYKTTPPVLDSDGSFFLYSALTVDKSRWQQGNVFSCSVMHEALHNHYTQKSLSLSPGK

SEQ ID NO: 17 - protein, 227 aa, artificial sequence
  D356C+T366S+L368A+Y407V+F405K+Q347R
DKTHTCPPCPAPELLGGPSVFLFPPKPKDTLMISRTPEVTCVVVDVSHEDPEVKFNWYVDGVEVHNAKTKPREEQYNSTYRVVSVLTVLHQDWLNGKEYKCKVSNKALPAPIEKTISKAKGQPREPRVYTLPPSRCELTKNQVSLSCAVKGFYPSDIAVEWESNGQPENNYKTTPPVLDSDGSFKLVSKLTVDKSRWQQGNVFSCSVMHEALHNHYTQKSLSLSPGK

SEQ ID NO: 18 - protein, 471 aa, artificial sequence
  Y349C+T366W+K409A+Q347R
EVQLLESGGGVVQPGRSLRLSCIASGFTFSSYPMTWVRQAPGKGLEWVASISYDGSYKYKADSMKGRLTISRDNSKNTLYLEMNSLTAEDTAVYYCARTAFFNAYDFWGQGTLVTVSSASTKGPSVGGGGSGGGGSEIVMTQSPATLSVSPGERATLSCRASQSVRSNLAWYQQKPGQAPRLLIYAASTRATGIPARFSGSGSGTEFTLTISSLQSEDFAVYYCQQYNEWFRTSGQGTKVEIKRDKTHTCPPCPAPELLGGPSVFLFPPKPKDTLMISRTPEVTCVVVDVSHENPEVKFNWYVDGVEVHNAKTKPREEQYNSTYRVVSVLTVLHQDWLNGKEYKCKVSNKALPAPIEKTISKAKGQPREPRVCTLPPSRDELTKNQVSLWCLVKGFYPSDIAVEWESNGQPENNYKTTPPVLDSDGSFFLYSALTVDKSRWQQGNVFSCSVMHEALHNHYTQKSLSLSPGK

SEQ ID NO: 19 - protein, 227 aa, artificial sequence
  D356C+T366S+L368A+Y407V+F405K+K360E+Q347E
DKTHTCPPCPAPELLGGPSVFLFPPKPKDTLMISRTPEVTCVVVDVSHEDPEVKFNWYVDGVEVHNAKTKPREEQYNSTYRVVSVLTVLHQDWLNGKEYKCKVSNKALPAPIEKTISKAKGQPREPEVYTLPPSRCELTENQVSLSCAVKGFYPSDIAVEWESNGQPENNYKTTPPVLDSDGSFKLVSKLTVDKSRWQQGNVFSCSVMHEALHNHYTQKSLSLSPGK

SEQ ID NO: 20 - protein, 471 aa, artificial sequence
  Y349C+T366W+K409A+L368E
EVQLLESGGGVVQPGRSLRLSCIASGFTFSSYPMTWVRQAPGKGLEWVASISYDGSYKYKADSMKGRLTISRDNSKNTLYLEMNSLTAEDTAVYYCARTAFFNAYDFWGQGTLVTVSSASTKGPSVGGGGSGGGGSEIVMTQSPATLSVSPGERATLSCRASQSVRSNLAWYQQKPGQAPRLLIYAASTRATGIPARFSGSGSGTEFTLTISSLQSEDFAVYYCQQYNEWFRTSGQGTKVEIKRDKTHTCPPCPAPELLGGPSVFLFPPKPKDTLMISRTPEVTCVVVDVSHENPEVKFNWYVDGVEVHNAKTKPREEQYNSTYRVVSVLTVLHQDWLNGKEYKCKVSNKALPAPIEKTISKAKGQPREPQVCTLPPSRDELTKNQVSLWCEVKGFYPSDIAVEWESNGQPENNYKTTPPVLDSDGSFFLYSALTVDKSRWQQGNVFSCSVMHEALHNHYTQKSLSLSPGK

SEQ ID NO: 21 - protein, 471 aa, artificial sequence
  T366W+K409A+K392D
EVQLLESGGGVVQPGRSLRLSCIASGFTFSSYPMTWVRQAPGKGLEWVASISYDGSYKYKADSMKGRLTISRDNSKNTLYLEMNSLTAEDTAVYYCARTAFFNAYDFWGQGTLVTVSSASTKGPSVGGGGSGGGGSEIVMTQSPATLSVSPGERATLSCRASQSVRSNLAWYQQKPGQAPRLLIYAASTRATGIPARFSGSGSGTEFTLTISSLQSEDFAVYYCQQYNEWFRTSGQGTKVEIKRDKTHTCPPCPAPELLGGPSVFLFPPKPKDTLMISRTPEVTCVVVDVSHENPEVKFNWYVDGVEVHNAKTKPREEQYNSTYRVVSVLTVLHQDWLNGKEYKCKVSNKALPAPIEKTISKAKGQPREPQVYTLPPSRDELTKNQVSLWCLVKGFYPSDIAVEWESNGQPENNYDTTPPVLDSDGSFFLYSALTVDKSRWQQGNVFSCSVMHEALHNHYTQKSLSLSPGK

SEQ ID NO: 22 - protein, 227 aa, artificial sequence
  T366S+L368A+Y407V+D399S+F405K
DKTHTCPPCPAPELLGGPSVFLFPPKPKDTLMISRTPEVTCVVVDVSHEDPEVKFNWYVDGVEVHNAKTKPREEQYNSTYRVVSVLTVLHQDWLNGKEYKCKVSNKALPAPIEKTISKAKGQPREPQVYTLPPSRDELTKNQVSLSCAVKGFYPSDIAVEWESNGQPENNYKTTPPVLSSDGSFKLVSKLTVDKSRWQQGNVFSCSVMHEALHNHYTQKSLSLSPGK

SEQ ID NO: 23 - protein, 471 aa, artificial sequence
  T366W+K409A
EVQLLESGGGVVQPGRSLRLSCIASGFTFSSYPMTWVRQAPGKGLEWVASISYDGSYKYKADSMKGRLTISRDNSKNTLYLEMNSLTAEDTAVYYCARTAFFNAYDFWGQGTLVTVSSASTKGPSVGGGGSGGGGSEIVMTQSPATLSVSPGERATLSCRASQSVRSNLAWYQQKPGQAPRLLIYAASTRATGIPARFSGSGSGTEFTLTISSLQSEDFAVYYCQQYNEWFRTSGQGTKVEIKRDKTHTCPPCPAPELLGGPSVFLFPPKPKDTLMISRTPEVTCVVVDVSHENPEVKFNWYVDGVEVHNAKTKPREEQYNSTYRVVSVLTVLHQDWLNGKEYKCKVSNKALPAPIEKTISKAKGQPREPQVYTLPPSRDELTKNQVSLWCLVKGFYPSDIAVEWESNGQPENNYKTTPPVLDSDGSFFLYSALTVDKSRWQQGNVFSCSVMHEALHNHYTQKSLSLSPGK

SEQ ID NO: 24 - protein, 227 aa, artificial sequence
  T366S+L368G+Y407A+F405K
DKTHTCPPCPAPELLGGPSVFLFPPKPKDTLMISRTPEVTCVVVDVSHEDPEVKFNWYVDGVEVHNAKTKPREEQYNSTYRVVSVLTVLHQDWLNGKEYKCKVSNKALPAPIEKTISKAKGQPREPQVYTLPPSRDELTKNQVSLSCGVKGFYPSDIAVEWESNGQPENNYKTTPPVLDSDGSFKLASKLTVDKSRWQQGNVFSCSVMHEALHNHYTQKSLSLSPGK

SEQ ID NO: 25 - protein, 227 aa, artificial sequence
  T366S+L368A+Y407V+F405K+E357A
DKTHTCPPCPAPELLGGPSVFLFPPKPKDTLMISRTPEVTCVVVDVSHEDPEVKFNWYVDGVEVHNAKTKPREEQYNSTYRVVSVLTVLHQDWLNGKEYKCKVSNKALPAPIEKTISKAKGQPREPQVYTLPPSRDALTKNQVSLSCAVKGFYPSDIAVEWESNGQPENNYKTTPPVLDSDGSFKLVSKLTVDKSRWQQGNVFSCSVMHEALHNHYTQKSLSLSPGK

SEQ ID NO: 26 - protein, 471 aa, artificial sequence
  T366W+K409A+Y349D+S354D
EVQLLESGGGVVQPGRSLRLSCIASGFTFSSYPMTWVRQAPGKGLEWVASISYDGSYKYKADSMKGRLTISRDNSKNTLYLEMNSLTAEDTAVYYCARTAFFNAYDFWGQGTLVTVSSASTKGPSVGGGGSGGGGSEIVMTQSPATLSVSPGERATLSCRASQSVRSNLAWYQQKPGQAPRLLIYAASTRATGIPARFSGSGSGTEFTLTISSLQSEDFAVYYCQQYNEWFRTSGQGTKVEIKRDKTHTCPPCPAPELLGGPSVFLFPPKPKDTLMISRTPEVTCVVVDVSHENPEVKFNWYVDGVEVHNAKTKPREEQYNSTYRVVSVLTVLHQDWLNGKEYKCKVSNKALPAPIEKTISKAKGQPREPQVDTLPPDRDELTKNQVSLWCLVKGFYPSDIAVEWESNGQPENNYKTTPPVLDSDGSFFLYSALTVDKSRWQQGNVFSCSVMHEALHNHYTQKSLSLSPGK

SEQ ID NO: 27 - protein, 471 aa, artificial sequence
  T366W+F405K
EVQLLESGGGVVQPGRSLRLSCIASGFTFSSYPMTWVRQAPGKGLEWVASISYDGSYKYKADSMKGRLTISRDNSKNTLYLEMNSLTAEDTAVYYCARTAFFNAYDFWGQGTLVTVSSASTKGPSVGGGGSGGGGSEIVMTQSPATLSVSPGERATLSCRASQSVRSNLAWYQQKPGQAPRLLIYAASTRATGIPARFSGSGSGTEFTLTISSLQSEDFAVYYCQQYNEWFRTSGQGTKVEIKRDKTHTCPPCPAPELLGGPSVFLFPPKPKDTLMISRTPEVTCVVVDVSHENPEVKFNWYVDGVEVHNAKTKPREEQYNSTYRVVSVLTVLHQDWLNGKEYKCKVSNKALPAPIEKTISKAKGQPREPQVYTLPPSRDELTKNQVSLWCLVKGFYPSDIAVEWESNGQPENNYKTTPPVLDSDGSFKLYSKLTVDKSRWQQGNVFSCSVMHEALHNHYTQKSLSLSPGK

SEQ ID NO: 28 - protein, 227 aa, artificial sequence
  T366S+L368A+Y407V+K409A
DKTHTCPPCPAPELLGGPSVFLFPPKPKDTLMISRTPEVTCVVVDVSHEDPEVKFNWYVDGVEVHNAKTKPREEQYNSTYRVVSVLTVLHQDWLNGKEYKCKVSNKALPAPIEKTISKAKGQPREPQVYTLPPSRDELTKNQVSLSCAVKGFYPSDIAVEWESNGQPENNYKTTPPVLDSDGSFFLVSALTVDKSRWQQGNVFSCSVMHEALHNHYTQKSLSLSPGK

SEQ ID NO: 29 - protein, 471 aa, artificial sequence
  T366W+F405K+D399S
EVQLLESGGGVVQPGRSLRLSCIASGFTFSSYPMTWVRQAPGKGLEWVASISYDGSYKYKADSMKGRLTISRDNSKNTLYLEMNSLTAEDTAVYYCARTAFFNAYDFWGQGTLVTVSSASTKGPSVGGGGSGGGGSEIVMTQSPATLSVSPGERATLSCRASQSVRSNLAWYQQKPGQAPRLLIYAASTRATGIPARFSGSGSGTEFTLTISSLQSEDFAVYYCQQYNEWFRTSGQGTKVEIKRDKTHTCPPCPAPELLGGPSVFLFPPKPKDTLMISRTPEVTCVVVDVSHENPEVKFNWYVDGVEVHNAKTKPREEQYNSTYRVVSVLTVLHQDWLNGKEYKCKVSNKALPAPIEKTISKAKGQPREPQVYTLPPSRDELTKNQVSLWCLVKGFYPSDIAVEWESNGQPENNYKTTPPVLSSDGSFKLYSKLTVDKSRWQQGNVFSCSVMHEALHNHYTQKSLSLSPGK

SEQ ID NO: 30 - protein, 227 aa, artificial sequence
  T366S+L368A+Y407V+K409A+K392D
DKTHTCPPCPAPELLGGPSVFLFPPKPKDTLMISRTPEVTCVVVDVSHEDPEVKFNWYVDGVEVHNAKTKPREEQYNSTYRVVSVLTVLHQDWLNGKEYKCKVSNKALPAPIEKTISKAKGQPREPQVYTLPPSRDELTKNQVSLSCAVKGFYPSDIAVEWESNGQPENNYDTTPPVLDSDGSFFLVSALTVDKSRWQQGNVFSCSVMHEALHNHYTQKSLSLSPGK

SEQ ID NO: 31 - protein, 227 aa, artificial sequence
  T366S+L368G+Y407A+K409A
DKTHTCPPCPAPELLGGPSVFLFPPKPKDTLMISRTPEVTCVVVDVSHEDPEVKFNWYVDGVEVHNAKTKPREEQYNSTYRVVSVLTVLHQDWLNGKEYKCKVSNKALPAPIEKTISKAKGQPREPQVYTLPPSRDELTKNQVSLSCGVKGFYPSDIAVEWESNGQPENNYKTTPPVLDSDGSFFLASALTVDKSRWQQGNVFSCSVMHEALHNHYTQKSLSLSPGK

SEQ ID NO: 32 - protein, 471 aa, artificial sequence
  T366W +F405K +Y349D
EVQLLESGGGVVQPGRSLRLSCIASGFTFSSYPMTWVRQAPGKGLEWVASISYDGSYKYKADSMKGRLTISRDNSKNTLYLEMNSLTAEDTAVYYCARTAFFNAYDFWGQGTLVTVSSASTKGPSVGGGGSGGGGSEIVMTQSPATLSVSPGERATLSCRASQSVRSNLAWYQQKPGQAPRLLIYAASTRATGIPARFSGSGSGTEFTLTISSLQSEDFAVYYCQQYNEWFRTSGQGTKVEIKRDKTHTCPPCPAPELLGGPSVFLFPPKPKDTLMISRTPEVTCVVVDVSHENPEVKFNWYVDGVEVHNAKTKPREEQYNSTYRVVSVLTVLHQDWLNGKEYKCKVSNKALPAPIEKTISKAKGQPREPQVDTLPPSRDELTKNQVSLWCLVKGFYPSDIAVEWESNGQPENNYKTTPPVLDSDGSFKLYSKLTVDKSRWQQGNVFSCSVMHEALHNHYTQKSLSLSPGK

SEQ ID NO: 33 - protein, 227 aa, artificial sequence
  T366S+L368A+Y407V +K409A +E357A
DKTHTCPPCPAPELLGGPSVFLFPPKPKDTLMISRTPEVTCVVVDVSHEDPEVKFNWYVDGVEVHNAKTKPREEQYNSTYRVVSVLTVLHQDWLNGKEYKCKVSNKALPAPIEKTISKAKGQPREPQVYTLPPSRDALTKNQVSLSCAVKGFYPSDIAVEWESNGQPENNYKTTPPVLDSDGSFFLVSALTVDKSRWQQGNVFSCSVMHEALHNHYTQKSLSLSPGK

SEQ ID NO: 34 - protein, 471 aa, artificial sequence
  T366W+F405K+Y349D+S354D
EVQLLESGGGVVQPGRSLRLSCIASGFTFSSYPMTWVRQAPGKGLEWVASISYDGSYKYKADSMKGRLTISRDNSKNTLYLEMNSLTAEDTAVYYCARTAFFNAYDFWGQGTLVTVSSASTKGPSVGGGGSGGGGSEIVMTQSPATLSVSPGERATLSCRASQSVRSNLAWYQQKPGQAPRLLIYAASTRATGIPARFSGSGSGTEFTLTISSLQSEDFAVYYCQQYNEWFRTSGQGTKVEIKRDKTHTCPPCPAPELLGGPSVFLFPPKPKDTLMISRTPEVTCVVVDVSHENPEVKFNWYVDGVEVHNAKTKPREEQYNSTYRVVSVLTVLHQDWLNGKEYKCKVSNKALPAPIEKTISKAKGQPREPQVDTLPPDRDELTKNQVSLWCLVKGFYPSDIAVEWESNGQPENNYKTTPPVLDSDGSFKLYSKLTVDKSRWQQGNVFSCSVMHEALHNHYTQKSLSLSPGK

SEQ ID NO: 35 - protein, 354 aa, artificial sequence
  VhH-Fc fusion protein
QVQLQESGGGSVQAGGSLRLSCAASEYIYSSYCMAWFRQAPGKEREGVAVIGSDGSTSYADSVKGRFTISKDNAKNTLYLQMNSLKPEDTAMYYCAAIGGYCYQPPYEYQYWGQGTQVTVSSEPKSSDKTHTCPPCPAPELLGGPSVFLFPPKPKDTLMISRTPEVTCVVVDVSHEDPEVKFNWYVDGVEVHNAKTKPREEQYNSTYRVVSVLTVLHQDWLNGKEYKCKVSNKALPAPIEKTISKAKGQPREPQVYTLPPSRDELTKNQVSLTCLVKGFYPSDIAVEWESNGQPENNYKTTPPVLDSDGSFFLYSKLTVDKSRWQQGNVFSCSVMHEALHNHYTQKSLSLSPGK

SEQ ID NO: 36 - DNA, 1121 bp, artificial sequence
  VhH-Fc encoding genes
atggagaccgacaccctgctgctgtgggtgctgctgctgtgggtgcccggcagcaccggccaggtgcagctgcaggagtctgggggaggctcggtgcaggctggagggtctctgagactctcctgtgcagcctctgaatacatctacagtagctactgcatggcctggttccgccaggctccagggaaggagcgcgagggggtcgcagttattgggagtgatggtagcacaagctacgcagactccgtgaaaggccgattcaccatctccaaagacaacgccaagaacactctgtatctgcaaatgaacagcctgaaacctgaggacactgccatgtactactgtgcggccatcggtggttactgctaccaaccaccctatgagtaccagtactggggccaggggacccaggtcaccgtctcccagaaccgaaaagcagcgacaagacccacacctgccccccctgccccgcccccgagctgctgggcggccccagcgtgttcctgttcccccccaagcccaaggacaccctgatgatcagccgcacccccgaggtgacctgcgtggtggtggacgtgagccacgagaaccccgaggtgaagttcaactggtacgtggacggcgtggaggtgcacaacgccaagaccaagccccgcgaggagcagtacaacagcacctaccgcgtggtgagcgtgctgaccgtgctgcaccaggactggctgaacggcaaggagtacaagtgcaaggtgagcaacaaggccctgcccgcccccatcgagaagaccatcagcaaggccaagggccagccccgcgagccccaggtgtacaccctgccccccagccgcgacgagctgaccaagaaccaggtgagcctgacctgcctggtgaagggcttctaccccagcgacatcgccgtggagtgggagagcaacggccagcccgagaacaactacaagaccaccccccccgtgctggacagcgacggcagcttcttcctgtacagcaagctgaccgtggacaagagccgctggcagcagggcaacgtgttcagctgcagcgtgatgcacgaggccctgcacaaccactacacccagaagagcctgagcctgagccccggcaag